European Patent Specification EP 2 539 465 B1, published March 6, 2024. Title: Analyte Sequencing with Nanopores. Applicant: University of Washington Gundlach, J.H. Derrington, I.M. Collins, M.D. The sequence listing filed with the application follows.

SEQUENCE LISTING (55 sequences)

SEQ ID NO: 1 - DNA, 4 bp, Artificial Sequence
  Synthetic
atgc

SEQ ID NO: 2 - DNA, 4 bp, Artificial Sequence
  Synthetic
tacg

SEQ ID NO: 3 - DNA, 5 bp, Artificial Sequence
  Synthetic
gtcac

SEQ ID NO: 4 - DNA, 84 bp, Artificial Sequence
  Synthetic
gctggctctgttgctctctcgcaacagagccagcaaaaaaaaaaaaaaaaaaaaaaaaaaaaaaaaaaaaaaaaaaaaaaaaaa

SEQ ID NO: 5 - DNA, 100 bp, Artificial Sequence
  Synthetic
gcaacagagccagccccgcaacagagccagcggagcaacagagccagctttgcaacagagccagcaaaaaaaaaaaaaaaaaaaaaaaaaaaaaaaaaaa

SEQ ID NO: 6 - DNA, 100 bp, Artificial Sequence
  Synthetic
gcaacagagccagcggagcaacagagccagccccgcaacagagccagcaaagcaacagagccagctttaaaaaaaaaaaaaaaaaaaaaaaaaaaaaaaa

SEQ ID NO: 7 - DNA, 100 bp, Artificial Sequence
  Synthetic
gcaacagagccagccccgcaacagagccagcaaagcaacagagccagccccgcaacagagccagctttgcaacagagccagcggaaaaaaaaaaaaaaaa

SEQ ID NO: 8 - DNA, 14 bp, Artificial Sequence
  Synthetic
gctggctctgttgc

SEQ ID NO: 9 - DNA, 180 bp, Artificial Sequence
  Synthetic
gctggctctgttgctctctcgcaacagagccagccccgctggctctgttgctctctcgcaacagagccagcggagctggctctgttgctctctcgcaacagagccagctttgctggctctgttgctctctcgcaacagagccagcaaaaaaaaaaaaaaaaaaaaaaaaaaaaaaaaaaa

SEQ ID NO: 10 - DNA, 50 bp, Artificial Sequence
  Synthetic
aaaaaaaaaaaaaaaaaaaaaaaaaaaaaaaaaaaaaaaaaaaaaaaaaa

SEQ ID NO: 11 - DNA, 50 bp, Artificial Sequence
  Synthetic
cccccccccccccccccccccccccccccccccccccccccccccccccc

SEQ ID NO: 12 - DNA, 50 bp, Artificial Sequence
  Synthetic
tttttttttttttttttttttttttttttttttttttttttttttttttt

SEQ ID NO: 13 - DNA, 47 bp, Artificial Sequence
  Synthetic
aaaaaaaaaaaaaaaaaaaaaaaaaaaaaaaaaaaaaaaaaaaaaaa

SEQ ID NO: 14 - DNA, 50 bp, Artificial Sequence
  Synthetic
gggggggggggggggggggggggggggggggggggggggggggggggggg

SEQ ID NO: 15 - DNA, 50 bp, Artificial Sequence
  Synthetic
caaaaaaaaaaaaaaaaaaaaaaaaaaaaaaaaaaaaaaaaaaaaaaaaa

SEQ ID NO: 16 - DNA, 50 bp, Artificial Sequence
  Synthetic
acaaaaaaaaaaaaaaaaaaaaaaaaaaaaaaaaaaaaaaaaaaaaaaaa

SEQ ID NO: 17 - DNA, 50 bp, Artificial Sequence
  Synthetic
aacaaaaaaaaaaaaaaaaaaaaaaaaaaaaaaaaaaaaaaaaaaaaaaa

SEQ ID NO: 18 - DNA, 50 bp, Artificial Sequence
  Synthetic
accaaaaaaaaaaaaaaaaaaaaaaaaaaaaaaaaaaaaaaaaaaaaaaa

SEQ ID NO: 19 - DNA, 50 bp, Artificial Sequence
  Synthetic
cacaaaaaaaaaaaaaaaaaaaaaaaaaaaaaaaaaaaaaaaaaaaaaaa

SEQ ID NO: 20 - DNA, 50 bp, Artificial Sequence
  Synthetic
ccaaaaaaaaaaaaaaaaaaaaaaaaaaaaaaaaaaaaaaaaaaaaaaaa

SEQ ID NO: 21 - DNA, 50 bp, Artificial Sequence
  Synthetic
taaaaaaaaaaaaaaaaaaaaaaaaaaaaaaaaaaaaaaaaaaaaaaaaa

SEQ ID NO: 22 - DNA, 50 bp, Artificial Sequence
  Synthetic
ataaaaaaaaaaaaaaaaaaaaaaaaaaaaaaaaaaaaaaaaaaaaaaaa

SEQ ID NO: 23 - DNA, 50 bp, Artificial Sequence
  Synthetic
aataaaaaaaaaaaaaaaaaaaaaaaaaaaaaaaaaaaaaaaaaaaaaaa

SEQ ID NO: 24 - DNA, 50 bp, Artificial Sequence
  Synthetic
attttttttttttttttttttttttttttttttttttttttttttttttt

SEQ ID NO: 25 - DNA, 50 bp, Artificial Sequence
  Synthetic
tatttttttttttttttttttttttttttttttttttttttttttttttt

SEQ ID NO: 26 - DNA, 50 bp, Artificial Sequence
  Synthetic
ttattttttttttttttttttttttttttttttttttttttttttttttt

SEQ ID NO: 27 - DNA, 50 bp, Artificial Sequence
  Synthetic
gggaaaaaaaaaaaaaaaaaaaaaaaaaaaaaaaaaaaaaaaaaaaaaaa

SEQ ID NO: 28 - DNA, 50 bp, Artificial Sequence
  Synthetic
ccccaaaaaaaaaaaaaaaaaaaaaaaaaaaaaaaaaaaaaaaaaaaaaa

SEQ ID NO: 29 - DNA, 50 bp, Artificial Sequence
  Synthetic
aaaccccaaaaaaaaaaaaaaaaaaaaaaaaaaaaaaaaaaaaaaaaaaa

SEQ ID NO: 30 - DNA, 50 bp, Artificial Sequence
  Synthetic
aaaaaaccccaaaaaaaaaaaaaaaaaaaaaaaaaaaaaaaaaaaaaaaa

SEQ ID NO: 31 - DNA, 50 bp, Artificial Sequence
  Synthetic
aaatacgcatacatcctaagaactcagactacctcccaataaatccacac

SEQ ID NO: 32 - DNA, 50 bp, Artificial Sequence
  Synthetic
aaatcagactacctcccaataaatccgcagcaatcctcacacctaataat

SEQ ID NO: 33 - DNA, 50 bp, Artificial Sequence
  Synthetic
ccctacgcatacatcctaagaactcagactacctcccaataaatccacac

SEQ ID NO: 34 - DNA, 50 bp, Artificial Sequence
  Synthetic
ccctcagactacctcccaataaatccgcagcaatcctcacacctaataat

SEQ ID NO: 35 - DNA, 50 bp, Artificial Sequence; identical to SEQ ID NO: 15
  Synthetic

SEQ ID NO: 36 - DNA, 50 bp, Artificial Sequence; identical to SEQ ID NO: 16
  Synthetic

SEQ ID NO: 37 - DNA, 50 bp, Artificial Sequence
  Synthetic
accccccccccccccccccccccccccccccccccccccccccccccccc

SEQ ID NO: 38 - DNA, 50 bp, Artificial Sequence
  Synthetic
cacccccccccccccccccccccccccccccccccccccccccccccccc

SEQ ID NO: 39 - DNA, 50 bp, Artificial Sequence; identical to SEQ ID NO: 21
  Synthetic

SEQ ID NO: 40 - DNA, 50 bp, Artificial Sequence; identical to SEQ ID NO: 22
  Synthetic

SEQ ID NO: 41 - DNA, 50 bp, Artificial Sequence; identical to SEQ ID NO: 24
  Synthetic

SEQ ID NO: 42 - DNA, 50 bp, Artificial Sequence; identical to SEQ ID NO: 25
  Synthetic

SEQ ID NO: 43 - DNA, 50 bp, Artificial Sequence
  Synthetic
gaaaaaaaaaaaaaaaaaaaaaaaaaaaaaaaaaaaaaaaaaaaaaaaaa

SEQ ID NO: 44 - DNA, 50 bp, Artificial Sequence
  Synthetic
agaaaaaaaaaaaaaaaaaaaaaaaaaaaaaaaaaaaaaaaaaaaaaaaa

SEQ ID NO: 45 - DNA, 50 bp, Artificial Sequence
  Synthetic
aagaaaaaaaaaaaaaaaaaaaaaaaaaaaaaaaaaaaaaaaaaaaaaaa

SEQ ID NO: 46 - DNA, 84 bp, Artificial Sequence
  Synthetic
tctggctctgttgctctctcgcaacagagccagaaaaaaaaaaaaaaaaaaaaaaaaaaaaaaaaaaaaaaaaaaaaaaaaaaa

SEQ ID NO: 47 - DNA, 84 bp, Artificial Sequence
  Synthetic
cctggctctgttgctctctcgcaacagagccaggaaaaaaaaaaaaaaaaaaaaaaaaaaaaaaaaaaaaaaaaaaaaaaaaaa

SEQ ID NO: 48 - DNA, 84 bp, Artificial Sequence
  Synthetic
actggctctgttgctctctcgcaacagagccagtaaaaaaaaaaaaaaaaaaaaaaaaaaaaaaaaaaaaaaaaaaaaaaaaaa

SEQ ID NO: 49 - DNA, 84 bp, Artificial Sequence
  Synthetic
gccggctctggtgctctctcgcaccagagccggcaaaaaaaaaaaaaaaaaaaaaaaaaaaaaaaaaaaaaaaaaaaaaaaaaa

SEQ ID NO: 50 - DNA, 80 bp, Artificial Sequence
  Synthetic
gctgtctgttgctctctcgcaacagacagcaaaaaaaaaaaaaaaaaaaaaaaaaaaaaaaaaaaaaaaaaaaaaaaaaa

SEQ ID NO: 51 - DNA, 76 bp, Artificial Sequence
  Synthetic
gctctgttgctctctcgcaacagagcaaaaaaaaaaaaaaaaaaaaaaaaaaaaaaaaaaaaaaaaaaaaaaaaaa

SEQ ID NO: 52 - DNA, 72 bp, Artificial Sequence
  Synthetic
gctgttgctctctcgcaacagcaaaaaaaaaaaaaaaaaaaaaaaaaaaaaaaaaaaaaaaaaaaaaaaaaa

SEQ ID NO: 53 - DNA, 100 bp, Artificial Sequence
  Synthetic
aaaaaaaaaaaaaaaaaaaaaaaaaaaaaaaaaaaaaaaaaaaaaaaaaaaaaaaaaaaaaaaaaaaaaaaaaaaaaaaaaaaaaaaaaaaaaaaaaaaa

SEQ ID NO: 54 - DNA, 50 bp, Artificial Sequence; identical to SEQ ID NO: 27
  Synthetic

SEQ ID NO: 55 - DNA, 4 bp, Artificial Sequence
  Synthetic
cccc